European Patent Application EP 4 403 574 A1, published July 24, 2024. Title: PROTEIN SPECIFICALLY BINDING TO PD-1 AND PHARMACEUTICAL USE THEREOF. Applicant: JIANGSU HENGRUI PHARMACEUTICALS CO., LTD. Application WO PCT/CN2022/118979, filed September 15, 2022. The sequence listing filed with the application follows.

SEQUENCE LISTING (101 sequences)

SEQ ID NO: 1 - protein, 288 aa, synthetic construct
MQIPQAPWPVVWAVLQLGWRPGWFLDSPDRPWNPPTFSPALLVVTEGDNATFTCSFSNTSESFVLNWYRMSPSNQTDKLAAFPEDRSQPGQDCRFRVTQLPNGRDFHMSVVRARRNDSGTYLCGAISLAPKAQIKESLRAELRVTERRAEVPTAHPSPSPRPAGQFQTLVVGVVGGLLGSLVLLVWVLAVICSRAARGTIGARRTGQPLKEDPSAVPVFSVDYGELDFQWREKTPEPPVPCVPEQTEYATIVFPSGMGTSSPARRGSADGPRSAQPLRPEDGHCSWPL

SEQ ID NO: 2 - protein, 122 aa, synthetic construct
EVQLVESGGGLVQAGGSLRLSCAVSGRTFSSAAMGWFRQAPGKEREFVAAISWSFGSTYYADSVKGRFTISRDNAKNTVYLQMNSLKPEDTAVYYCAADPSIETMGGGWDYWGQGTQVTVSS

SEQ ID NO: 3 - protein, 116 aa, synthetic construct
EVQVVESGGGLVQPGGSLRLSCVASGLTFSDYSMSWYRQAPGKERELVAIISGSGVIAHYVDSVKGRFTISRDNAKSTVYLQMVSLKPEDRGVYYCRAVSDWDDYWGQGTQVTVSS

SEQ ID NO: 4 - protein, 5 aa, synthetic construct
SAAMG

SEQ ID NO: 5 - protein, 16 aa, synthetic construct
ISWSFGSTYYADSVKG

SEQ ID NO: 6 - protein, 13 aa, synthetic construct
DPSIETMGGGWDY

SEQ ID NO: 7 - protein, 5 aa, synthetic construct
DYSMS

SEQ ID NO: 8 - protein, 17 aa, synthetic construct
IISGSGVIAHYVDSVKG

SEQ ID NO: 9 - protein, 7 aa, synthetic construct
VSDWDDY

SEQ ID NO: 10 - protein, 229 aa, synthetic construct
ESKYGPPCPPCPAPEFLGGPSVFLFPPKPKDTLMISRTPEVTCVVVDVSQEDPEVQFNWYVDGVEVHNAKTKPREEQFNSTYRVVSVLTVLHQDWLNGKEYKCKVSNKGLPSSIEKTISKAKGQPREPQVYTLPPSQEEMTKNQVSLTCLVKGFYPSDIAVEWESNGQPENNYKTTPPVLDSDGSFFLYSRLTVDKSRWQEGNVFSCSVMHEALHNHYTQKSLSLSLGK

SEQ ID NO: 11 - protein, 351 aa, synthetic construct
EVQLVESGGGLVQAGGSLRLSCAVSGRTFSSAAMGWFRQAPGKEREFVAAISWSFGSTYYADSVKGRFTISRDNAKNTVYLQMNSLKPEDTAVYYCAADPSIETMGGGWDYWGQGTQVTVSSESKYGPPCPPCPAPEFLGGPSVFLFPPKPKDTLMISRTPEVTCVVVDVSQEDPEVQFNWYVDGVEVHNAKTKPREEQFNSTYRVVSVLTVLHQDWLNGKEYKCKVSNKGLPSSIEKTISKAKGQPREPQVYTLPPSQEEMTKNQVSLTCLVKGFYPSDIAVEWESNGQPENNYKTTPPVLDSDGSFFLYSRLTVDKSRWQEGNVFSCSVMHEALHNHYTQKSLSLSLGK

SEQ ID NO: 12 - protein, 345 aa, synthetic construct
EVQVVESGGGLVQPGGSLRLSCVASGLTFSDYSMSWYRQAPGKERELVAIISGSGVIAHYVDSVKGRFTISRDNAKSTVYLQMVSLKPEDRGVYYCRAVSDWDDYWGQGTQVTVSSESKYGPPCPPCPAPEFLGGPSVFLFPPKPKDTLMISRTPEVTCVVVDVSQEDPEVQFNWYVDGVEVHNAKTKPREEQFNSTYRVVSVLTVLHQDWLNGKEYKCKVSNKGLPSSIEKTISKAKGQPREPQVYTLPPSQEEMTKNQVSLTCLVKGFYPSDIAVEWESNGQPENNYKTTPPVLDSDGSFFLYSRLTVDKSRWQEGNVFSCSVMHEALHNHYTQKSLSLSLGK

SEQ ID NO: 13 - protein, 116 aa, synthetic construct
EVQLQESGGGLVQPGGSLRLSCTASGLTFSDYSMSWYRQAPGKGRELVAIISGSGVIAHYVDSVKGRFTISRDNSKNTVYLQMRSLTPEDRAVYYCRAVSDWDDYWGQGTQVTVSS

SEQ ID NO: 14 - protein, 116 aa, synthetic construct
EVQLVESGGGLVQPGGSLRLSCAASGLTFSDYSMSWVRQAPGKGLEWVAIISGSGVIAHYVDSVKGRFTISRDNSKNTVYLQMNSLRAEDTAVYYCRAVSDWDDYWGQGTQVTVSS

SEQ ID NO: 15 - protein, 116 aa, synthetic construct
EVQLVESGGGLVQPGGSLRLSCAASGLTFSDYSMSWVRQAPGKGLEWVAIISGSGVIAHYVDSVKGRFTISRDNSKNTVYLQMNSLRAEDTAVYYCRAVSDWDEYWGQGTQVTVSS

SEQ ID NO: 16 - protein, 122 aa, synthetic construct
EVQLLESGGGLVQAGGSLRLSCATSGRTFSSAAMGWFRQAPGKGLEWVAAISWSFGSTYYADSVKGRFTISRDNSKNTVYLQMNSLRPEDTAVYYCAADPSIETMGGGWDYWGQGTQVTVSS

SEQ ID NO: 17 - protein, 116 aa, synthetic construct
EVQLQESGGGLVQPGGSLRLSCTASGLTFSDYSMSWYRQAPGKGRELVAIISGSGVIAHYVDSVKGRFTISRDNAKNTVYLQMRSLTPEDRAVYYCRAVSDWDDYWGQGTQVTVSS

SEQ ID NO: 18 - protein, 116 aa, synthetic construct
EVQLQESGGGLVQPGGSLRLSCTASGLTFSDYSMSWYRQAPGKGRELVAIISGSGVITHYVDSVKGRFTISRDNSKNTVYLQMRSLTPEDRAVYYCRAVSDWDDYWGQGTQVTVSS

SEQ ID NO: 19 - protein, 116 aa, synthetic construct
EVQLQESGGGLVQPGGSLRLSCTASGLTFSDYSMSWYRQAPGKGRELVAIISGSGGIAHYVDSVKGRFTISRDNSKNTVYLQMRSLTPEDRAVYYCRAVSDWDDYWGQGTQVTVSS

SEQ ID NO: 20 - protein, 116 aa, synthetic construct
EVQLQESGGGLVQPGGSLRLSCTASGLTFSDYSMSWYRQAPGKGRELVAIISGSGVSAHYVDSVKGRFTISRDNSKNTVYLQMRSLTPEDRAVYYCRAVSDWDDYWGQGTQVTVSS

SEQ ID NO: 21 - protein, 116 aa, synthetic construct
EVQLQESGGGLVQPGGSLRLSCTASGLTFSDYSMSWYRQAPGKGRELVAIISGSGVIAHYVDSVKGRFTISRDNSKNTVYLQMRSLTPEDRAVYYCRAVSDWEDYWGQGTQVTVSS

SEQ ID NO: 22 - protein, 116 aa, synthetic construct
EVQLQESGGGLVQPGGSLRLSCTASGLTFSDYSMSWYRQAPGKGRELVAIISGSGVIAHYVDSVKGRFTISRDNSKNTVYLQMRSLTPEDRAVYYCRAVSDWDEYWGQGTQVTVSS

SEQ ID NO: 23 - protein, 116 aa, synthetic construct
EVQLQESGGGLVQPGGSLRLSCTASGLTFSDYSMSWYRQAPGKGRELVAIISGSGVIAHYVDSVKGRFTISRDNAKNTVYLQMRSLTPEDRAVYYCRAVSDWEDYWGQGTQVTVSS

SEQ ID NO: 24 - protein, 116 aa, synthetic construct
EVQLQESGGGLVQPGGSLRLSCTASGLTFSDYSMSWYRQAPGKGRELVAIISGSGVIAHYVDSVKGRFTISRDNAKNTVYLQMRSLTPEDRAVYYCRAVSDWDEYWGQGTQVTVSS

SEQ ID NO: 25 - protein, 116 aa, synthetic construct
EVQLQESGGGLVQPGGSLRLSCTASGLTFSDYSMSWYRQAPGKGRELVAIISGSGVITHYVDSVKGRFTISRDNAKNTVYLQMRSLTPEDRAVYYCRAVSDWEDYWGQGTQVTVSS

SEQ ID NO: 26 - protein, 116 aa, synthetic construct
EVQLQESGGGLVQPGGSLRLSCTASGLTFSDYSMSWYRQAPGKGRELVAIISGSGVITHYVDSVKGRFTISRDNAKNTVYLQMRSLTPEDRAVYYCRAVSDWDEYWGQGTQVTVSS

SEQ ID NO: 27 - protein, 116 aa, synthetic construct
EVQLQESGGGLVQPGGSLRLSCTASGLTFSDYSMSWYRQAPGKGRELVAIISGSGGIAHYVDSVKGRFTISRDNAKNTVYLQMRSLTPEDRAVYYCRAVSDWEDYWGQGTQVTVSS

SEQ ID NO: 28 - protein, 116 aa, synthetic construct
EVQLQESGGGLVQPGGSLRLSCTASGLTFSDYSMSWYRQAPGKGRELVAIISGSGGIAHYVDSVKGRFTISRDNAKNTVYLQMRSLTPEDRAVYYCRAVSDWDEYWGQGTQVTVSS

SEQ ID NO: 29 - protein, 116 aa, synthetic construct
EVQLQESGGGLVQPGGSLRLSCTASGLTFSDYSMSWYRQAPGKGRELVAIISGSGVSAHYVDSVKGRFTISRDNAKNTVYLQMRSLTPEDRAVYYCRAVSDWEDYWGQGTQVTVSS

SEQ ID NO: 30 - protein, 116 aa, synthetic construct
EVQLQESGGGLVQPGGSLRLSCTASGLTFSDYSMSWYRQAPGKGRELVAIISGSGVSAHYVDSVKGRFTISRDNAKNTVYLQMRSLTPEDRAVYYCRAVSDWDEYWGQGTQVTVSS

SEQ ID NO: 31 - protein, 116 aa, synthetic construct
EVQLQESGGGLVQPGGSLRLSCTASGLTFSDYSMSWYRQAPGKGRELVAIISGSGGITHYVDSVKGRFTISRDNAKNTVYLQMRSLTPEDRAVYYCRAVSDWEDYWGQGTQVTVSS

SEQ ID NO: 32 - protein, 116 aa, synthetic construct
EVQLVESGGGLVQPGGSLRLSCAASGFTFSDYSMSWYRQAPGKGRELVAIISGSGVITHYVDSVKGRFTISRDNAKNTLYLQMRSLRAEDTAVYYCRAVSDWEDYWGQGTQVTVSS

SEQ ID NO: 33 - protein, 116 aa, synthetic construct
EVQLVESGGGLVQPGGSLRLSCAASGLTFSDYSMSWYRQAPGKGRELVAIISGSGVITHYVDSVKGRFTISRDNAKNTLYLQMRSLRAEDTAVYYCRAVSDWEDYWGQGTQVTVSS

SEQ ID NO: 34 - protein, 116 aa, synthetic construct
EVQLVESGGGLVQPGGSLRLSCAASGLTFSDYSMSWYRQAPGKGRELVAIISGSGVITHYVDSVKGRFTISRDNAKNTVYLQMRSLRAEDTAVYYCRAVSDWEDYWGQGTQVTVSS

SEQ ID NO: 35 - protein, 116 aa, synthetic construct
EVQLVESGGGLVQPGGSLRLSCAASGLTFSDYSMSWYRQAPGKGRELVAIISGSGVITHYVDSVKGRFTISRDNAKNTVYLQMRSLRAEDRAVYYCRAVSDWEDYWGQGTQVTVSS

SEQ ID NO: 36 - protein, 17 aa, synthetic construct
  VARIANT 7: note = X is V or G; note (original language) = X is selected from the group consisting of V and G
  VARIANT 9: note = X is T or A; note (original language) = X is selected from the group consisting of T and A
  VARIANT 8: note = X is I or S; note (original language) = X is selected from the group consisting of I and S
IISGSGXXXHYVDSVKG

SEQ ID NO: 37 - protein, 7 aa, synthetic construct
  VARIANT 5: note = X is D or E; note (original language) = X is selected from the group consisting of D and E
  VARIANT 6: note = X is D or E; note (original language) = X is selected from the group consisting of D and E
VSDWXXY

SEQ ID NO: 38 - protein, 17 aa, synthetic construct
IISGSGVITHYVDSVKG

SEQ ID NO: 39 - protein, 17 aa, synthetic construct
IISGSGGIAHYVDSVKG

SEQ ID NO: 40 - protein, 17 aa, synthetic construct
IISGSGVSAHYVDSVKG

SEQ ID NO: 41 - protein, 7 aa, synthetic construct
VSDWEDY

SEQ ID NO: 42 - protein, 7 aa, synthetic construct
VSDWDEY

SEQ ID NO: 43 - protein, 137 aa, synthetic construct
TPEVWVQVQMEATELSSFTVHCGFLGPGSISLVTVSWGGPDGAGGTKLAVLHPELGTRQWAPARQARWETQSSISLALEDSGASSPFANTTFCCKFASFPEGSWESCGSLPPSSDPGLSAPPTPVPILRADHHHHHH

SEQ ID NO: 44 - protein, 121 aa, synthetic construct
HVQLVESGGGSVQAGGSLRLSCEASGYSYSGDCMGWFRRAPGKERDEGVATIDNAGRIKYADSVKGRFTISHGNGKYILYLQMNSLKPEDTDMYYCAAGWTFGGNCSPADWGQGTQVTVSS

SEQ ID NO: 45 - protein, 127 aa, synthetic construct
HVQLVESGGGSVQAGGSLRLSCVASASGFTYRPYCMAWFRQAPGKEREAVAGIDIFGGTTYADSVKGRFTASRDNAGFSLFLQMNDLKPEDTAMYYCAAGDSPDGRCPPLGQGLNYWGQGTQVTVSS

SEQ ID NO: 46 - protein, 5 aa, synthetic construct
GDCMG

SEQ ID NO: 47 - protein, 16 aa, synthetic construct
TIDNAGRIKYADSVKG

SEQ ID NO: 48 - protein, 12 aa, synthetic construct
GWTFGGNCSPAD

SEQ ID NO: 49 - protein, 7 aa, synthetic construct
YRPYCMA

SEQ ID NO: 50 - protein, 16 aa, synthetic construct
GIDIFGGTTYADSVKG

SEQ ID NO: 51 - protein, 17 aa, synthetic construct
GDSPDGRCPPLGQGLNY

SEQ ID NO: 52 - protein, 229 aa, synthetic construct
ESKYGPPCPPCPAPEAAGGPSVFLFPPKPKDTLMISRTPEVTCVVVDVSQEDPEVQFNWYVDGVEVHNAKTKPREEQFNSTYRVVSVLTVLHQDWLNGKEYKCKVSNKGLPSSIEKTISKAKGQPREPQVYTLPPSQEEMTKNQVSLTCLVKGFYPSDIAVEWESNGQPENNYKTTPPVLDSDGSFFLYSRLTVDKSRWQEGNVFSCSVMHEALHNHYTQKSLSLSLGA

SEQ ID NO: 53 - protein, 350 aa, synthetic construct
HVQLVESGGGSVQAGGSLRLSCEASGYSYSGDCMGWFRRAPGKERDEGVATIDNAGRIKYADSVKGRFTISHGNGKYILYLQMNSLKPEDTDMYYCAAGWTFGGNCSPADWGQGTQVTVSSESKYGPPCPPCPAPEAAGGPSVFLFPPKPKDTLMISRTPEVTCVVVDVSQEDPEVQFNWYVDGVEVHNAKTKPREEQFNSTYRVVSVLTVLHQDWLNGKEYKCKVSNKGLPSSIEKTISKAKGQPREPQVYTLPPSQEEMTKNQVSLTCLVKGFYPSDIAVEWESNGQPENNYKTTPPVLDSDGSFFLYSRLTVDKSRWQEGNVFSCSVMHEALHNHYTQKSLSLSLGA

SEQ ID NO: 54 - protein, 356 aa, synthetic construct
HVQLVESGGGSVQAGGSLRLSCVASASGFTYRPYCMAWFRQAPGKEREAVAGIDIFGGTTYADSVKGRFTASRDNAGFSLFLQMNDLKPEDTAMYYCAAGDSPDGRCPPLGQGLNYWGQGTQVTVSSESKYGPPCPPCPAPEAAGGPSVFLFPPKPKDTLMISRTPEVTCVVVDVSQEDPEVQFNWYVDGVEVHNAKTKPREEQFNSTYRVVSVLTVLHQDWLNGKEYKCKVSNKGLPSSIEKTISKAKGQPREPQVYTLPPSQEEMTKNQVSLTCLVKGFYPSDIAVEWESNGQPENNYKTTPPVLDSDGSFFLYSRLTVDKSRWQEGNVFSCSVMHEALHNHYTQKSLSLSLGA

SEQ ID NO: 55 - protein, 449 aa, synthetic construct
EVQLVESGGGVVKPGGSLRLSCAASGFTFGTSSMNWVRQAPGKGLEWVAVISFDGTEIHYADSVKGRFTISRDNSKSTVFLQMNSLRPDDTALYYCAKGSGNIYFYSGMDVWGQGTTVTVSSASTKGPSVFPLAPCSRSTSESTAALGCLVKDYFPEPVTVSWNSGALTSGVHTFPAVLQSSGLYSLSSVVTVPSSSLGTKTYTCNVDHKPSNTKVDKRVESKYGPPCPPCPAPEAAGGPSVFLFPPKPKDTLMISRTPEVTCVVVDVSQEDPEVQFNWYVDGVEVHNAKTKPREEQFNSTYRVVSVLTVLHQDWLNGKEYKCKVSNKGLPSSIEKTISKAKGQPREPQVYTLPPSQEEMTKNQVSLTCLVKGFYPSDIAVEWESNGQPENNYKTTPPVLDSDGSFFLYSRLTVDKSRWQEGNVFSCSVMHEALHNHYTQKSLSLSLGA

SEQ ID NO: 56 - protein, 214 aa, synthetic construct
DIQMTQSPSTLSASVGDRVTITCRAGQSISGWLAWFQQKPGKAPNLLIYETSTLESGVPSRFSGSGSGTEYTLTISSLQPDDFATYYCQQYYSYPLTFGQGTKVEIKRTVAAPSVFIFPPSDEQLKSGTASVVCLLNNFYPREAKVQWKVDNALQSGNSQESVTEQDSKDSTYSLSSTLTLSKADYEKHKVYACEVTHQGLSSPVTKSFNRGEC

SEQ ID NO: 57 - protein, 120 aa, synthetic construct
EVQLVESGGGLVQPGGSLRLSCAASGFTFSGDCMGWFRQAPGKGLEGVATIDNAGRIKYADSVKGRFTISRDNAKNSLYLQMNSLRAEDTAVYYCAAGWTFGGQCSPADWGQGTQVTVSS

SEQ ID NO: 58 - protein, 121 aa, synthetic construct
EVQLVESGGGLVQPGGSLRLSCAASGFTFSGDCMGWFRQAPGKGLDEGVATIDNAGRIKYADSVKGRFTISRDNAKNSLYLQMNSLRAEDTAVYYCAAGWTFGGQCSPADWGQGTQVTVSS

SEQ ID NO: 59 - protein, 121 aa, synthetic construct
EVQLVESGGGLVQPGGSLRLSCAASGYSYSGDCMGWFRQAPGKGLDEGVATIDNAGRIKYADSVKGRFTISRDNAKNSLYLQMNSLRAEDTAVYYCAAGWTFGGQCSPADWGQGTQVTVSS

SEQ ID NO: 60 - protein, 121 aa, synthetic construct
EVQLVESGGGLVQPGGSLRLSCAASGFTFSGDCMGWFRQAPGKGLDEGVATIDNAGRIKYADSVKGRFTISHGNAKYILYLQMNSLRAEDTAVYYCAAGWTFGGQCSPADWGQGTQVTVSS

SEQ ID NO: 61 - protein, 121 aa, synthetic construct
EVQLVESGGGLVQPGGSLRLSCAASGYSYSGDCMGWFRQAPGKGLDEGVATIDNAGRIKYADSVKGRFTISHGNAKYILYLQMNSLRAEDTAVYYCAAGWTFGGQCSPADWGQGTQVTVSS

SEQ ID NO: 62 - protein, 125 aa, synthetic construct
EVQLVESGGGLVQPGGSLRLSCAASGFTYRPYCMAWFRQAPGKGLEAVAGIDIFGGTTYADSVKGRFTISRDNAKNSLYLQMNSLRAEDTAVYYCAAGDSPDGRCPPLGQGLNYWGQGTMVTVSS

SEQ ID NO: 63 - protein, 127 aa, synthetic construct
EVQLVESGGGLVQPGGSLRLSCVASASGFTYRPYCMAWFRQAPGKGLEAVAGIDIFGGTTYADSVKGRFTISRDNAKNSLYLQMNSLRAEDTAVYYCAAGDSPDGRCPPLGQGLNYWGQGTMVTVSS

SEQ ID NO: 64 - protein, 127 aa, synthetic construct
HVQLVESGGGLVQPGGSLRLSCVASASGFTYRPYCMAWFRQAPGKEREAVAGIDIFGGTTYADSVKGRFTASRDNAGFSLYLQMNSLRAEDTAVYYCAAGDSPDGRCPPLGQGLNYWGQGTMVTVSS

SEQ ID NO: 65 - protein, 127 aa, synthetic construct
EVQLVESGGGLVQPGGSLRLSCVASASGFTYRPYCMAWFRQAPGKGLEAVAGIDIFGGTTYADSVKGRFTISRDNAGFSLYLQMNSLRAEDTAVYYCAAGDSPDGRCPPLGQGLNYWGQGTMVTVSS

SEQ ID NO: 66 - protein, 127 aa, synthetic construct
HVQLVESGGGLVQPGGSLRLSCVASASGFTYRPYCMAWFRQAPGKGLEAVAGIDIFGGTTYADSVKGRFTASRDNAGFSLYLQMNSLRAEDTAVYYCAAGDSPDGRCPPLGQGLNYWGQGTMVTVSS

SEQ ID NO: 67 - protein, 446 aa, synthetic construct
EVQLVQSGAEVKKPGASVKVSCKASGYTFTNYWMHWVRQAPGQGLEWMGRIDPDSTGSKYNEKFKTRVTMTRDTSTSTVYMELSSLRSEDTAVYYCAREGAYGYYFDYWGQGTLVTVSSASTKGPSVFPLAPCSRSTSESTAALGCLVKDYFPEPVTVSWNSGALTSGVHTFPAVLQSSGLYSLSSVVTVPSSSLGTKTYTCNVDHKPSNTKVDKRVESKYGPPCPPCPAPEFLGGPSVFLFPPKPKDTLMISRTPEVTCVVVDVSQEDPEVQFNWYVDGVEVHNAKTKPREEQFNSTYRVVSVLTVLHQDWLNGKEYKCKVSNKGLPSSIEKTISKAKGQPREPQVYTLPPSQEEMTKNQVSLTCLVKGFYPSDIAVEWESNGQPENNYKTTPPVLDSDGSFFLYSRLTVDKSRWQEGNVFSCSVMHEALHNHYTQKSLSLSLGK

SEQ ID NO: 68 - protein, 214 aa, synthetic construct
DIQMTQSPSSLSASVGDRVTITCRASENIYSYLAWYQQKPGKSPKLLIYNARTLAEGVPSRFSGSGSGTDFTLTISSLQPEDFATYYCQYHSGSPLPFGGGTKVEIKRTVAAPSVFIFPPSDEQLKSGTASVVCLLNNFYPREAKVQWKVDNALQSGNSQESVTEQDSKDSTYSLSSTLTLSKADYEKHKVYACEVTHQGLSSPVTKSFNRGEC

SEQ ID NO: 69 - protein, 583 aa, synthetic construct
HVQLVESGGGSVQAGGSLRLSCVASASGFTYRPYCMAWFRQAPGKEREAVAGIDIFGGTTYADSVKGRFTASRDNAGFSLFLQMNDLKPEDTAMYYCAAGDSPDGRCPPLGQGLNYWGQGTQVTVSSGGGGSGGGGSEVQLVQSGAEVKKPGASVKVSCKASGYTFTNYWMHWVRQAPGQGLEWMGRIDPDSTGSKYNEKFKTRVTMTRDTSTSTVYMELSSLRSEDTAVYYCAREGAYGYYFDYWGQGTLVTVSSASTKGPSVFPLAPCSRSTSESTAALGCLVKDYFPEPVTVSWNSGALTSGVHTFPAVLQSSGLYSLSSVVTVPSSSLGTKTYTCNVDHKPSNTKVDKRVESKYGPPCPPCPAPEFLGGPSVFLFPPKPKDTLMISRTPEVTCVVVDVSQEDPEVQFNWYVDGVEVHNAKTKPREEQFNSTYRVVSVLTVLHQDWLNGKEYKCKVSNKGLPSSIEKTISKAKGQPREPQVYTLPPSQEEMTKNQVSLTCLVKGFYPSDIAVEWESNGQPENNYKTTPPVLDSDGSFFLYSRLTVDKSRWQEGNVFSCSVMHEALHNHYTQKSLSLSLGK

SEQ ID NO: 70 - protein, 583 aa, synthetic construct
EVQLVQSGAEVKKPGASVKVSCKASGYTFTNYWMHWVRQAPGQGLEWMGRIDPDSTGSKYNEKFKTRVTMTRDTSTSTVYMELSSLRSEDTAVYYCAREGAYGYYFDYWGQGTLVTVSSASTKGPSVFPLAPCSRSTSESTAALGCLVKDYFPEPVTVSWNSGALTSGVHTFPAVLQSSGLYSLSSVVTVPSSSLGTKTYTCNVDHKPSNTKVDKRVESKYGPPCPPCPAPEFLGGPSVFLFPPKPKDTLMISRTPEVTCVVVDVSQEDPEVQFNWYVDGVEVHNAKTKPREEQFNSTYRVVSVLTVLHQDWLNGKEYKCKVSNKGLPSSIEKTISKAKGQPREPQVYTLPPSQEEMTKNQVSLTCLVKGFYPSDIAVEWESNGQPENNYKTTPPVLDSDGSFFLYSRLTVDKSRWQEGNVFSCSVMHEALHNHYTQKSLSLSLGKGGGGSGGGGSHVQLVESGGGSVQAGGSLRLSCVASASGFTYRPYCMAWFRQAPGKEREAVAGIDIFGGTTYADSVKGRFTASRDNAGFSLFLQMNDLKPEDTAMYYCAAGDSPDGRCPPLGQGLNYWGQGTQVTVSS

SEQ ID NO: 71 - protein, 351 aa, synthetic construct
HVQLVESGGGSVQAGGSLRLSCVASASGFTYRPYCMAWFRQAPGKEREAVAGIDIFGGTTYADSVKGRFTASRDNAGFSLFLQMNDLKPEDTAMYYCAAGDSPDGRCPPLGQGLNYWGQGTQVTVSSGGGGSGGGGSDIQMTQSPSSLSASVGDRVTITCRASENIYSYLAWYQQKPGKSPKLLIYNARTLAEGVPSRFSGSGSGTDFTLTISSLQPEDFATYYCQYHSGSPLPFGGGTKVEIKRTVAAPSVFIFPPSDEQLKSGTASVVCLLNNFYPREAKVQWKVDNALQSGNSQESVTEQDSKDSTYSLSSTLTLSKADYEKHKVYACEVTHQGLSSPVTKSFNRGEC

SEQ ID NO: 72 - protein, 351 aa, synthetic construct
DIQMTQSPSSLSASVGDRVTITCRASENIYSYLAWYQQKPGKSPKLLIYNARTLAEGVPSRFSGSGSGTDFTLTISSLQPEDFATYYCQYHSGSPLPFGGGTKVEIKRTVAAPSVFIFPPSDEQLKSGTASVVCLLNNFYPREAKVQWKVDNALQSGNSQESVTEQDSKDSTYSLSSTLTLSKADYEKHKVYACEVTHQGLSSPVTKSFNRGECGGGGSGGGGSHVQLVESGGGSVQAGGSLRLSCVASASGFTYRPYCMAWFRQAPGKEREAVAGIDIFGGTTYADSVKGRFTASRDNAGFSLFLQMNDLKPEDTAMYYCAAGDSPDGRCPPLGQGLNYWGQGTQVTVSS

SEQ ID NO: 73 - protein, 5 aa, synthetic construct
NYWMH

SEQ ID NO: 74 - protein, 17 aa, synthetic construct
RIDPDSTGSKYNEKFKT

SEQ ID NO: 75 - protein, 10 aa, synthetic construct
EGAYGYYFDY

SEQ ID NO: 76 - protein, 11 aa, synthetic construct
RASENIYSYLA

SEQ ID NO: 77 - protein, 7 aa, synthetic construct
NARTLAE

SEQ ID NO: 78 - protein, 9 aa, synthetic construct
QYHSGSPLP

SEQ ID NO: 79 - protein, 119 aa, synthetic construct
EVQLVQSGAEVKKPGASVKVSCKASGYTFTNYWMHWVRQAPGQGLEWMGRIDPDSTGSKYNEKFKTRVTMTRDTSTSTVYMELSSLRSEDTAVYYCAREGAYGYYFDYWGQGTLVTVSS

SEQ ID NO: 80 - protein, 119 aa, synthetic construct
EVQLVQSGAEVKKPGASVKVSCKASGYTFTNYWMHWVRQAPGQGLEWMGRIDPDSTGSKYNEKFKTRVTMTVDTSTSTVYMELSSLRSEDTAVYYCAREGAYGYYFDYWGQGTLVTVSS

SEQ ID NO: 81 - protein, 119 aa, synthetic construct
EVQLVQSGAEVKKPGASVKVSCKASGYTFTNYWMHWVRQAPGQGLEWIGRIDPDSTGSKYNEKFKTRVTMTVDTSTSTAYMELSSLRSEDTAVYYCAREGAYGYYFDYWGQGTLVTVSS

SEQ ID NO: 82 - protein, 107 aa, synthetic construct
DIQMTQSPSSLSASVGDRVTITCRASENIYSYLAWYQQKPGKAPKLLIYNARTLAEGVPSRFSGSGSGTDFTLTISSLQPEDFATYYCQYHSGSPLPFGGGTKVEIK

SEQ ID NO: 83 - protein, 107 aa, synthetic construct
DIQMTQSPSSLSASVGDRVTITCRASENIYSYLAWYQQKPGKSPKLLIYNARTLAEGVPSRFSGSGSGTDFTLTISSLQPEDFATYYCQYHSGSPLPFGGGTKVEIK

SEQ ID NO: 84 - protein, 577 aa, synthetic construct
EVQLVESGGGLVQPGGSLRLSCAASGFTFSGDCMGWFRQAPGKGLDEGVATIDNAGRIKYADSVKGRFTISRDNAKNSLYLQMNSLRAEDTAVYYCAAGWTFGGQCSPADWGQGTQVTVSSGGGGSGGGGSEVQLVQSGAEVKKPGASVKVSCKASGYTFTNYWMHWVRQAPGQGLEWMGRIDPDSTGSKYNEKFKTRVTMTRDTSTSTVYMELSSLRSEDTAVYYCAREGAYGYYFDYWGQGTLVTVSSASTKGPSVFPLAPCSRSTSESTAALGCLVKDYFPEPVTVSWNSGALTSGVHTFPAVLQSSGLYSLSSVVTVPSSSLGTKTYTCNVDHKPSNTKVDKRVESKYGPPCPPCPAPEFLGGPSVFLFPPKPKDTLMISRTPEVTCVVVDVSQEDPEVQFNWYVDGVEVHNAKTKPREEQFNSTYRVVSVLTVLHQDWLNGKEYKCKVSNKGLPSSIEKTISKAKGQPREPQVYTLPPSQEEMTKNQVSLTCLVKGFYPSDIAVEWESNGQPENNYKTTPPVLDSDGSFFLYSRLTVDKSRWQEGNVFSCSVMHEALHNHYTQKSLSLSLGK

SEQ ID NO: 85 - protein, 583 aa, synthetic construct
HVQLVESGGGLVQPGGSLRLSCVASASGFTYRPYCMAWFRQAPGKEREAVAGIDIFGGTTYADSVKGRFTASRDNAGFSLYLQMNSLRAEDTAVYYCAAGDSPDGRCPPLGQGLNYWGQGTMVTVSSGGGGSGGGGSEVQLVQSGAEVKKPGASVKVSCKASGYTFTNYWMHWVRQAPGQGLEWMGRIDPDSTGSKYNEKFKTRVTMTRDTSTSTVYMELSSLRSEDTAVYYCAREGAYGYYFDYWGQGTLVTVSSASTKGPSVFPLAPCSRSTSESTAALGCLVKDYFPEPVTVSWNSGALTSGVHTFPAVLQSSGLYSLSSVVTVPSSSLGTKTYTCNVDHKPSNTKVDKRVESKYGPPCPPCPAPEFLGGPSVFLFPPKPKDTLMISRTPEVTCVVVDVSQEDPEVQFNWYVDGVEVHNAKTKPREEQFNSTYRVVSVLTVLHQDWLNGKEYKCKVSNKGLPSSIEKTISKAKGQPREPQVYTLPPSQEEMTKNQVSLTCLVKGFYPSDIAVEWESNGQPENNYKTTPPVLDSDGSFFLYSRLTVDKSRWQEGNVFSCSVMHEALHNHYTQKSLSLSLGK

SEQ ID NO: 86 - protein, 583 aa, synthetic construct
EVQLVESGGGLVQPGGSLRLSCVASASGFTYRPYCMAWFRQAPGKGLEAVAGIDIFGGTTYADSVKGRFTISRDNAGFSLYLQMNSLRAEDTAVYYCAAGDSPDGRCPPLGQGLNYWGQGTMVTVSSGGGGSGGGGSEVQLVQSGAEVKKPGASVKVSCKASGYTFTNYWMHWVRQAPGQGLEWMGRIDPDSTGSKYNEKFKTRVTMTRDTSTSTVYMELSSLRSEDTAVYYCAREGAYGYYFDYWGQGTLVTVSSASTKGPSVFPLAPCSRSTSESTAALGCLVKDYFPEPVTVSWNSGALTSGVHTFPAVLQSSGLYSLSSVVTVPSSSLGTKTYTCNVDHKPSNTKVDKRVESKYGPPCPPCPAPEFLGGPSVFLFPPKPKDTLMISRTPEVTCVVVDVSQEDPEVQFNWYVDGVEVHNAKTKPREEQFNSTYRVVSVLTVLHQDWLNGKEYKCKVSNKGLPSSIEKTISKAKGQPREPQVYTLPPSQEEMTKNQVSLTCLVKGFYPSDIAVEWESNGQPENNYKTTPPVLDSDGSFFLYSRLTVDKSRWQEGNVFSCSVMHEALHNHYTQKSLSLSLGK

SEQ ID NO: 87 - protein, 703 aa, synthetic construct
EVQLVESGGGLVQPGGSLRLSCAASGLTFSDYSMSWYRQAPGKGRELVAIISGSGVITHYVDSVKGRFTISRDNAKNTLYLQMRSLRAEDTAVYYCRAVSDWEDYWGQGTQVTVSSGGGGSGGGGSEVQLVESGGGLVQPGGSLRLSCAASGFTFSGDCMGWFRQAPGKGLDEGVATIDNAGRIKYADSVKGRFTISRDNAKNSLYLQMNSLRAEDTAVYYCAAGWTFGGQCSPADWGQGTQVTVSSGGGGSGGGGSEVQLVQSGAEVKKPGASVKVSCKASGYTFTNYWMHWVRQAPGQGLEWMGRIDPDSTGSKYNEKFKTRVTMTRDTSTSTVYMELSSLRSEDTAVYYCAREGAYGYYFDYWGQGTLVTVSSASTKGPSVFPLAPCSRSTSESTAALGCLVKDYFPEPVTVSWNSGALTSGVHTFPAVLQSSGLYSLSSVVTVPSSSLGTKTYTCNVDHKPSNTKVDKRVESKYGPPCPPCPAPEFLGGPSVFLFPPKPKDTLMISRTPEVTCVVVDVSQEDPEVQFNWYVDGVEVHNAKTKPREEQFNSTYRVVSVLTVLHQDWLNGKEYKCKVSNKGLPSSIEKTISKAKGQPREPQVYTLPPSQEEMTKNQVSLTCLVKGFYPSDIAVEWESNGQPENNYKTTPPVLDSDGSFFLYSRLTVDKSRWQEGNVFSCSVMHEALHNHYTQKSLSLSLGK

SEQ ID NO: 88 - protein, 340 aa, synthetic construct
EVQLVESGGGLVQPGGSLRLSCAASGLTFSDYSMSWYRQAPGKGRELVAIISGSGVITHYVDSVKGRFTISRDNAKNTLYLQMRSLRAEDTAVYYCRAVSDWEDYWGQGTQVTVSSGGGGSGGGGSDIQMTQSPSSLSASVGDRVTITCRASENIYSYLAWYQQKPGKSPKLLIYNARTLAEGVPSRFSGSGSGTDFTLTISSLQPEDFATYYCQYHSGSPLPFGGGTKVEIKRTVAAPSVFIFPPSDEQLKSGTASVVCLLNNFYPREAKVQWKVDNALQSGNSQESVTEQDSKDSTYSLSSTLTLSKADYEKHKVYACEVTHQGLSSPVTKSFNRGEC

SEQ ID NO: 89 - protein, 703 aa, synthetic construct
EVQLVESGGGLVQPGGSLRLSCAASGFTFSGDCMGWFRQAPGKGLDEGVATIDNAGRIKYADSVKGRFTISRDNAKNSLYLQMNSLRAEDTAVYYCAAGWTFGGQCSPADWGQGTQVTVSSGGGGSGGGGSEVQLVQSGAEVKKPGASVKVSCKASGYTFTNYWMHWVRQAPGQGLEWMGRIDPDSTGSKYNEKFKTRVTMTRDTSTSTVYMELSSLRSEDTAVYYCAREGAYGYYFDYWGQGTLVTVSSASTKGPSVFPLAPCSRSTSESTAALGCLVKDYFPEPVTVSWNSGALTSGVHTFPAVLQSSGLYSLSSVVTVPSSSLGTKTYTCNVDHKPSNTKVDKRVESKYGPPCPPCPAPEFLGGPSVFLFPPKPKDTLMISRTPEVTCVVVDVSQEDPEVQFNWYVDGVEVHNAKTKPREEQFNSTYRVVSVLTVLHQDWLNGKEYKCKVSNKGLPSSIEKTISKAKGQPREPQVYTLPPSQEEMTKNQVSLTCLVKGFYPSDIAVEWESNGQPENNYKTTPPVLDSDGSFFLYSRLTVDKSRWQEGNVFSCSVMHEALHNHYTQKSLSLSLGKGGGGSGGGGSEVQLVESGGGLVQPGGSLRLSCAASGLTFSDYSMSWYRQAPGKGRELVAIISGSGVITHYVDSVKGRFTISRDNAKNTLYLQMRSLRAEDTAVYYCRAVSDWEDYWGQGTQVTVSS

SEQ ID NO: 90 - protein, 340 aa, synthetic construct
DIQMTQSPSSLSASVGDRVTITCRASENIYSYLAWYQQKPGKSPKLLIYNARTLAEGVPSRFSGSGSGTDFTLTISSLQPEDFATYYCQYHSGSPLPFGGGTKVEIKRTVAAPSVFIFPPSDEQLKSGTASVVCLLNNFYPREAKVQWKVDNALQSGNSQESVTEQDSKDSTYSLSSTLTLSKADYEKHKVYACEVTHQGLSSPVTKSFNRGECGGGGSGGGGSEVQLVESGGGLVQPGGSLRLSCAASGLTFSDYSMSWYRQAPGKGRELVAIISGSGVITHYVDSVKGRFTISRDNAKNTLYLQMRSLRAEDTAVYYCRAVSDWEDYWGQGTQVTVSS

SEQ ID NO: 91 - protein, 709 aa, synthetic construct
EVQLVESGGGLVQPGGSLRLSCAASGLTFSDYSMSWYRQAPGKGRELVAIISGSGVITHYVDSVKGRFTISRDNAKNTLYLQMRSLRAEDTAVYYCRAVSDWEDYWGQGTQVTVSSGGGGSGGGGSHVQLVESGGGLVQPGGSLRLSCVASASGFTYRPYCMAWFRQAPGKEREAVAGIDIFGGTTYADSVKGRFTASRDNAGFSLYLQMNSLRAEDTAVYYCAAGDSPDGRCPPLGQGLNYWGQGTMVTVSSGGGGSGGGGSEVQLVQSGAEVKKPGASVKVSCKASGYTFTNYWMHWVRQAPGQGLEWMGRIDPDSTGSKYNEKFKTRVTMTRDTSTSTVYMELSSLRSEDTAVYYCAREGAYGYYFDYWGQGTLVTVSSASTKGPSVFPLAPCSRSTSESTAALGCLVKDYFPEPVTVSWNSGALTSGVHTFPAVLQSSGLYSLSSVVTVPSSSLGTKTYTCNVDHKPSNTKVDKRVESKYGPPCPPCPAPEFLGGPSVFLFPPKPKDTLMISRTPEVTCVVVDVSQEDPEVQFNWYVDGVEVHNAKTKPREEQFNSTYRVVSVLTVLHQDWLNGKEYKCKVSNKGLPSSIEKTISKAKGQPREPQVYTLPPSQEEMTKNQVSLTCLVKGFYPSDIAVEWESNGQPENNYKTTPPVLDSDGSFFLYSRLTVDKSRWQEGNVFSCSVMHEALHNHYTQKSLSLSLGK

SEQ ID NO: 92 - protein, 340 aa, synthetic construct; identical to SEQ ID NO: 88

SEQ ID NO: 93 - protein, 709 aa, synthetic construct
HVQLVESGGGLVQPGGSLRLSCVASASGFTYRPYCMAWFRQAPGKEREAVAGIDIFGGTTYADSVKGRFTASRDNAGFSLYLQMNSLRAEDTAVYYCAAGDSPDGRCPPLGQGLNYWGQGTMVTVSSGGGGSGGGGSEVQLVQSGAEVKKPGASVKVSCKASGYTFTNYWMHWVRQAPGQGLEWMGRIDPDSTGSKYNEKFKTRVTMTRDTSTSTVYMELSSLRSEDTAVYYCAREGAYGYYFDYWGQGTLVTVSSASTKGPSVFPLAPCSRSTSESTAALGCLVKDYFPEPVTVSWNSGALTSGVHTFPAVLQSSGLYSLSSVVTVPSSSLGTKTYTCNVDHKPSNTKVDKRVESKYGPPCPPCPAPEFLGGPSVFLFPPKPKDTLMISRTPEVTCVVVDVSQEDPEVQFNWYVDGVEVHNAKTKPREEQFNSTYRVVSVLTVLHQDWLNGKEYKCKVSNKGLPSSIEKTISKAKGQPREPQVYTLPPSQEEMTKNQVSLTCLVKGFYPSDIAVEWESNGQPENNYKTTPPVLDSDGSFFLYSRLTVDKSRWQEGNVFSCSVMHEALHNHYTQKSLSLSLGKGGGGSGGGGSEVQLVESGGGLVQPGGSLRLSCAASGLTFSDYSMSWYRQAPGKGRELVAIISGSGVITHYVDSVKGRFTISRDNAKNTLYLQMRSLRAEDTAVYYCRAVSDWEDYWGQGTQVTVSS

SEQ ID NO: 94 - protein, 340 aa, synthetic construct; identical to SEQ ID NO: 90

SEQ ID NO: 95 - protein, 127 aa, synthetic construct
EVQLVESGGGLVQPGGSLRLSCVASASGFTYRPYCMAWFRQAPGKEREAVAGIDIFGGTTYADSVKGRFTASRDNAGFSLYLQMNSLRAEDTAVYYCAAGDSPDGRCPPLGQGLNYWGQGTMVTVSS

SEQ ID NO: 96 - protein, 127 aa, synthetic construct
QVQLVESGGGLVQPGGSLRLSCVASASGFTYRPYCMAWFRQAPGKEREAVAGIDIFGGTTYADSVKGRFTASRDNAGFSLYLQMNSLRAEDTAVYYCAAGDSPDGRCPPLGQGLNYWGQGTMVTVSS

SEQ ID NO: 97 - protein, 709 aa, synthetic construct
EVQLVESGGGLVQPGGSLRLSCVASASGFTYRPYCMAWFRQAPGKEREAVAGIDIFGGTTYADSVKGRFTASRDNAGFSLYLQMNSLRAEDTAVYYCAAGDSPDGRCPPLGQGLNYWGQGTMVTVSSGGGGSGGGGSEVQLVQSGAEVKKPGASVKVSCKASGYTFTNYWMHWVRQAPGQGLEWMGRIDPDSTGSKYNEKFKTRVTMTRDTSTSTVYMELSSLRSEDTAVYYCAREGAYGYYFDYWGQGTLVTVSSASTKGPSVFPLAPCSRSTSESTAALGCLVKDYFPEPVTVSWNSGALTSGVHTFPAVLQSSGLYSLSSVVTVPSSSLGTKTYTCNVDHKPSNTKVDKRVESKYGPPCPPCPAPEFLGGPSVFLFPPKPKDTLMISRTPEVTCVVVDVSQEDPEVQFNWYVDGVEVHNAKTKPREEQFNSTYRVVSVLTVLHQDWLNGKEYKCKVSNKGLPSSIEKTISKAKGQPREPQVYTLPPSQEEMTKNQVSLTCLVKGFYPSDIAVEWESNGQPENNYKTTPPVLDSDGSFFLYSRLTVDKSRWQEGNVFSCSVMHEALHNHYTQKSLSLSLGKGGGGSGGGGSEVQLVESGGGLVQPGGSLRLSCAASGLTFSDYSMSWYRQAPGKGRELVAIISGSGVITHYVDSVKGRFTISRDNAKNTLYLQMRSLRAEDTAVYYCRAVSDWEDYWGQGTQVTVSS

SEQ ID NO: 98 - protein, 709 aa, synthetic construct
QVQLVESGGGLVQPGGSLRLSCVASASGFTYRPYCMAWFRQAPGKEREAVAGIDIFGGTTYADSVKGRFTASRDNAGFSLYLQMNSLRAEDTAVYYCAAGDSPDGRCPPLGQGLNYWGQGTMVTVSSGGGGSGGGGSEVQLVQSGAEVKKPGASVKVSCKASGYTFTNYWMHWVRQAPGQGLEWMGRIDPDSTGSKYNEKFKTRVTMTRDTSTSTVYMELSSLRSEDTAVYYCAREGAYGYYFDYWGQGTLVTVSSASTKGPSVFPLAPCSRSTSESTAALGCLVKDYFPEPVTVSWNSGALTSGVHTFPAVLQSSGLYSLSSVVTVPSSSLGTKTYTCNVDHKPSNTKVDKRVESKYGPPCPPCPAPEFLGGPSVFLFPPKPKDTLMISRTPEVTCVVVDVSQEDPEVQFNWYVDGVEVHNAKTKPREEQFNSTYRVVSVLTVLHQDWLNGKEYKCKVSNKGLPSSIEKTISKAKGQPREPQVYTLPPSQEEMTKNQVSLTCLVKGFYPSDIAVEWESNGQPENNYKTTPPVLDSDGSFFLYSRLTVDKSRWQEGNVFSCSVMHEALHNHYTQKSLSLSLGKGGGGSGGGGSEVQLVESGGGLVQPGGSLRLSCAASGLTFSDYSMSWYRQAPGKGRELVAIISGSGVITHYVDSVKGRFTISRDNAKNTLYLQMRSLRAEDTAVYYCRAVSDWEDYWGQGTQVTVSS

SEQ ID NO: 99 - protein, 12 aa, synthetic construct
GWTFGGQCSPAD

SEQ ID NO: 100 - protein, 10 aa, synthetic construct
GGGGSGGGGS

SEQ ID NO: 101 - protein, 17 aa, synthetic construct
IISGSGGITHYVDSVKG